European Patent Application EP 4 190 816 A1, published June 7, 2023. Title: ANTI-CD47 MONOCLONAL ANTIBODY AND USE THEREOF. Applicant: Akeso Biopharma, Inc AKESO PHARMACEUTICALS, INC. The sequence listing filed with the application follows.

SEQUENCE LISTING (146 sequences)

SEQ ID NO: 1 - DNA, 351 bp, Artificial Sequence
  Synthetic artificial sequence-Nucleotide sequence of the heavy chain variable region of 6F7
caggtgcagctgcagcagccaggagcagagctggtgaggccaggagcatccgtgaagctgtcttgtaaggccagcggctacaccttcacatcctattggatgaactgggtgaagcagaggcctggacagggactggagtggatcggcatgatcgacccaagcgattccgagacccacaacaatcagatgtttaaggacaaggccaccctgacagtggataagagctccaataccgcctacatgcacctgtctagcctgacatctgaggacagcgccgtgtatcactgcgcccggctgtacagatggtattttgacgtgtggggagcaggaaccacagtgaccgtgtcctct

SEQ ID NO: 2 - protein, 117 aa, Artificial Sequence
  Synthetic artificial sequence-Amino acid sequence of the heavy chain variable region of 6F7
QVQLQQPGAELVRPGASVKLSCKASGYTFTSYWMNWVKQRPGQGLEWIGMIDPSDSETHNNQMFKDKATLTVDKSSNTAYMHLSSLTSEDSAVYHCARLYRWYFDVWGAGTTVTVSS

SEQ ID NO: 3 - DNA, 321 bp, Artificial Sequence
  Synthetic artificial sequence-Nucleotide sequence of the variable region of the light chain of 6F7
aacatcgtgatgacccagtcccccaagtctatgagcatgtccctgggcgagagggtgaccctgtcctgtaaggcctctgagatcgtgggcacatacgtgtcttggtttcagcagaagccacaccagagccccaagctgctgatctacggcgcctccaatcggtatacaggcgtgcctgacagattcaccggctctggcagcgccacagacttcaccctgacaatctctaacgtgcaggccgaggacctggccgattatcactgcggccagagctacaatttcccttatacctttggcggcggcacaaagctggagatcaag

SEQ ID NO: 4 - protein, 107 aa, Artificial Sequence
  Synthetic artificial sequence-Amino acid sequence of the variable region of the light chain of 6F7
NIVMTQSPKSMSMSLGERVTLSCKASEIVGTYVSWFQQKPHQSPKLLIYGASNRYTGVPDRFTGSGSATDFTLTISNVQAEDLADYHCGQSYNFPYTFGGGTKLEIK

SEQ ID NO: 5 - protein, 8 aa, Artificial Sequence
  Synthetic artificial sequence-Amino acid sequence of HCDR1 of 6F7
GYTFTSYW

SEQ ID NO: 6 - protein, 8 aa, Artificial Sequence
  Synthetic artificial sequence-Amino acid sequence of HCDR2 of 6F7
IDPSDSET

SEQ ID NO: 7 - protein, 10 aa, Artificial Sequence
  Synthetic artificial sequence-Amino acid sequence of HCDR3 of 6F7
ARLYRWYFDV

SEQ ID NO: 8 - protein, 6 aa, Artificial Sequence
  Synthetic artificial sequence-Amino acid sequence of LCDR1 of 6F7
EIVGTY

SEQ ID NO: 9 - protein, 3 aa, Artificial Sequence
  Synthetic artificial sequence-Amino acid sequence of LCDR2 of 6F7
GAS

SEQ ID NO: 10 - protein, 9 aa, Artificial Sequence
  Synthetic artificial sequence-Amino acid sequence of LCDR3 of 6F7
GQSYNFPYT

SEQ ID NO: 11 - DNA, 351 bp, Artificial Sequence
  Synthetic artificial sequence-Nucleotide sequence of the heavy chain variable region of 6F7H1
caggtgcagctggtgcagagcggagcagaggtggtgaagccaggagcctctgtgaagctgagctgtaaggcctccggctacaccttcacaagctattggatgaactgggtgcggcagagaccaggacagggactggagtggatcggaatgatcgacccttccgattctgagacccacaatgcccagaagtttcagggcaaggccaccctgacagtggacaagagcacctccacagcctacatgcacctgagctccctgcggtccgaggacacagccgtgtactattgcgccaggctgtaccgctggtattttgacgtgtggggagcaggaaccacagtgaccgtgtctagc

SEQ ID NO: 12 - protein, 117 aa, Artificial Sequence
  Synthetic artificial sequence-Amino acid sequence of the heavy chain variable region of 6F7H1
QVQLVQSGAEVVKPGASVKLSCKASGYTFTSYWMNWVRQRPGQGLEWIGMIDPSDSETHNAQKFQGKATLTVDKSTSTAYMHLSSLRSEDTAVYYCARLYRWYFDVWGAGTTVTVSS

SEQ ID NO: 13 - DNA, 321 bp, Artificial Sequence
  Synthetic artificial sequence-Nucleotide sequence of the variable region of the light chain of 6F7L1
aacatcgtgatgacccagtccccagccacaatgtctatgagcccaggagagagggtgaccctgtcctgtagagcctctgagatcgtgggcacatacgtgtcttggtttcagcagaagccaggacaggcacctaggctgctgatctacggagcaagcaacaggtataccggagtgccagcacgcttctccggctctggcagcggcacagactttaccctgacaatcagctccgtgcagcctgaggacctggccgattatcactgcggccagtcttacaatttcccatatacctttggcggcggcacaaagctggagatcaag

SEQ ID NO: 14 - protein, 107 aa, Artificial Sequence
  Synthetic artificial sequence-Amino acid sequence of the variable region of the light chain of 6F7L1
NIVMTQSPATMSMSPGERVTLSCRASEIVGTYVSWFQQKPGQAPRLLIYGASNRYTGVPARFSGSGSGTDFTLTISSVQPEDLADYHCGQSYNFPYTFGGGTKLEIK

SEQ ID NO: 15 - DNA, 351 bp, Artificial Sequence
  Synthetic artificial sequence-Nucleotide sequence of the heavy chain variable region of 6F7H2
caggtgcagctggtgcagagcggagcagaggtggtgaagccaggagcctctgtgaaggtgagctgtaaggcctccggctacaccttcacatcctattggatgaactgggtgcggcagagaccaggacagggactggagtggatcggaatcatcgacccttccgattctgagacctctaatgcccagaagtttcagggccgggtgaccctgacagtggacaagagcacctccacagcctacatgcacctgagctccctgaggagcgaggacacagccgtgtactattgcgccaggctgtaccgctggtattttgacgtgtggggagcaggaaccacagtgaccgtgtctagc

SEQ ID NO: 16 - protein, 117 aa, Artificial Sequence
  Synthetic artificial sequence-Amino acid sequence of the heavy chain variable region of 6F7H2
QVQLVQSGAEVVKPGASVKVSCKASGYTFTSYWMNWVRQRPGQGLEWIGIIDPSDSETSNAQKFQGRVTLTVDKSTSTAYMHLSSLRSEDTAVYYCARLYRWYFDVWGAGTTVTVSS

SEQ ID NO: 17 - DNA, 321 bp, Artificial Sequence
  Synthetic artificial sequence-Nucleotide sequence of the variable region of the light chain of 6F7L2
aacatcgtgatgacccagtccccagccacactgtctctgagcccaggagagagggtgaccctgtcctgtagagcctctgagatcgtgggcacatacgtgtcttggtttcagcagaagccaggacaggcacctaggctgctgatctatggcgccagcaacagggcaaccggcatccccgcacgcttctccggctctggcagcggcacagactttaccctgacaatcagctccctgcagcctgaggacctggccgattactattgcggccagtcttacaatttcccatatacctttggcggcggcacaaagctggagatcaag

SEQ ID NO: 18 - protein, 107 aa, Artificial Sequence
  Synthetic artificial sequence-Amino acid sequence of the variable region of the light chain of 6F7L2
NIVMTQSPATLSLSPGERVTLSCRASEIVGTYVSWFQQKPGQAPRLLIYGASNRATGIPARFSGSGSGTDFTLTISSLQPEDLADYYCGQSYNFPYTFGGGTKLEIK

SEQ ID NO: 19 - DNA, 351 bp, Artificial Sequence
  Synthetic artificial sequence-Nucleotide sequence of the heavy chain variable region of 6F7H3
caggtgcagctggtgcagagcggagcagaggtggtgaagccaggagcctctgtgaaggtgagctgtaaggcctccggctacaccttcacatcctattggatgaactgggtgcggcaggcaccaggacagggactggagtggatcggcatcatcgacccttccgattctgagacctcttacgcccagaagtttcagggcagggtgaccctgacagtggacaagagcacctccacagcctatatggagctgagctccctgcgcagcgaggacacagccgtgtactattgcgcccggctgtacagatggtattttgacgtgtggggagcaggaaccacagtgaccgtgtctagc

SEQ ID NO: 20 - protein, 117 aa, Artificial Sequence
  Synthetic artificial sequence-Amino acid sequence of the heavy chain variable region of 6F7H3
QVQLVQSGAEVVKPGASVKVSCKASGYTFTSYWMNWVRQAPGQGLEWIGIIDPSDSETSYAQKFQGRVTLTVDKSTSTAYMELSSLRSEDTAVYYCARLYRWYFDVWGAGTTVTVSS

SEQ ID NO: 21 - DNA, 321 bp, Artificial Sequence
  Synthetic artificial sequence-Nucleotide sequence of the variable region of the light chain of 6F7L3
aacatcgtgatgacccagtccccagccacactgtctctgagcccaggagagagggtgaccctgtcctgtagagcctctgagatcgtgggcacatacctgtcttggtatcagcagaagccaggacaggcacctaggctgctgatctacggagccagcaccagggcaacaggcatccccgcacgcttctccggctctggcagcggcaccgactttaccctgacaatcagctccctgcagcctgaggattttgccgtgtactattgcggccagtcttacaatttcccatatacctttggcggcggcacaaagctggagatcaag

SEQ ID NO: 22 - protein, 107 aa, Artificial Sequence
  Synthetic artificial sequence-Amino acid sequence of the variable region of the light chain of 6F7L3
NIVMTQSPATLSLSPGERVTLSCRASEIVGTYLSWYQQKPGQAPRLLIYGASTRATGIPARFSGSGSGTDFTLTISSLQPEDFAVYYCGQSYNFPYTFGGGTKLEIK

SEQ ID NO: 23 - protein, 25 aa, Artificial Sequence
  Synthetic artificial sequence-FR-H1 amino acid sequence of the heavy chain skeleton region of 6F7
QVQLQQPGAELVRPGASVKLSCKAS

SEQ ID NO: 24 - protein, 17 aa, Artificial Sequence
  Synthetic artificial sequence-FR-H2 amino acid sequence of the heavy chain skeleton region of 6F7
MNWVKQRPGQGLEWIGM

SEQ ID NO: 25 - protein, 38 aa, Artificial Sequence
  Synthetic artificial sequence-FR-H3 amino acid sequence of the heavy chain skeleton region of 6F7
HNNQMFKDKATLTVDKSSNTAYMHLSSLTSEDSAVYHC

SEQ ID NO: 26 - protein, 11 aa, Artificial Sequence
  Synthetic artificial sequence-FR-H4 amino acid sequence of the heavy chain skeleton region of 6F7
WGAGTTVTVSS

SEQ ID NO: 27 - protein, 26 aa, Artificial Sequence
  Synthetic artificial sequence-FR-L1 amino acid sequence of 6F7 light chain skeleton
NIVMTQSPKSMSMSLGERVTLSCKAS

SEQ ID NO: 28 - protein, 17 aa, Artificial Sequence
  Synthetic artificial sequence-FR-L2 amino acid sequence of 6F7 light chain skeleton
VSWFQQKPHQSPKLLIY

SEQ ID NO: 29 - protein, 36 aa, Artificial Sequence
  Synthetic artificial sequence-FR-L3 amino acid sequence of 6F7 light chain skeleton
NRYTGVPDRFTGSGSATDFTLTISNVQAEDLADYHC

SEQ ID NO: 30 - protein, 10 aa, Artificial Sequence
  Synthetic artificial sequence-FR-L4 amino acid sequence of 6F7 light chain skeleton
FGGGTKLEIK

SEQ ID NO: 31 - protein, 25 aa, Artificial Sequence
  Synthetic artificial sequence-FR-H1 amino acid sequence of 6F7H1 skeleton region
QVQLVQSGAEVVKPGASVKLSCKAS

SEQ ID NO: 32 - protein, 17 aa, Artificial Sequence
  Synthetic artificial sequence-FR-H2 amino acid sequence of 6F7H1 skeleton region
MNWVRQRPGQGLEWIGM

SEQ ID NO: 33 - protein, 38 aa, Artificial Sequence
  Synthetic artificial sequence-FR-H3 amino acid sequence of 6F7H1 skeleton region
HNAQKFQGKATLTVDKSTSTAYMHLSSLRSEDTAVYYC

SEQ ID NO: 34 - protein, 11 aa, Artificial Sequence
  Synthetic artificial sequence-FR-H4 amino acid sequence of 6F7H1 skeleton region
WGAGTTVTVSS

SEQ ID NO: 35 - protein, 26 aa, Artificial Sequence
  Synthetic artificial sequence-FR-L1 amino acid sequence of 6F7L1 skeleton region
NIVMTQSPATMSMSPGERVTLSCRAS

SEQ ID NO: 36 - protein, 17 aa, Artificial Sequence
  Synthetic artificial sequence-FR-L2 amino acid sequence of 6F7L1 skeleton region
VSWFQQKPGQAPRLLIY

SEQ ID NO: 37 - protein, 36 aa, Artificial Sequence
  Synthetic artificial sequence-FR-L3 amino acid sequence of 6F7L1 skeleton region
NRYTGVPARFSGSGSGTDFTLTISSVQPEDLADYHC

SEQ ID NO: 38 - protein, 10 aa, Artificial Sequence
  Synthetic artificial sequence-FR-L4 amino acid sequence of 6F7L1 skeleton region
FGGGTKLEIK

SEQ ID NO: 39 - protein, 25 aa, Artificial Sequence
  Synthetic artificial sequence-FR-H1 amino acid sequence of 6F7H2 skeleton region
QVQLVQSGAEVVKPGASVKVSCKAS

SEQ ID NO: 40 - protein, 17 aa, Artificial Sequence
  Synthetic artificial sequence-FR-H2 amino acid sequence of 6F7H2 skeleton region
MNWVRQRPGQGLEWIGI

SEQ ID NO: 41 - protein, 38 aa, Artificial Sequence
  Synthetic artificial sequence-FR-H3 amino acid sequence of 6F7H2 skeleton region
SNAQKFQGRVTLTVDKSTSTAYMHLSSLRSEDTAVYYC

SEQ ID NO: 42 - protein, 11 aa, Artificial Sequence
  Synthetic artificial sequence-FR-H4 amino acid sequence of 6F7H2 skeleton region
WGAGTTVTVSS

SEQ ID NO: 43 - protein, 26 aa, Artificial Sequence
  Synthetic artificial sequence-FR-L1 amino acid sequence of 6F7L2 skeleton region
NIVMTQSPATLSLSPGERVTLSCRAS

SEQ ID NO: 44 - protein, 17 aa, Artificial Sequence
  Synthetic artificial sequence-FR-L2 amino acid sequence of 6F7L2 skeleton region
VSWFQQKPGQAPRLLIY

SEQ ID NO: 45 - protein, 36 aa, Artificial Sequence
  Synthetic artificial sequence-FR-L3 amino acid sequence of 6F7L2 skeleton region
NRATGIPARFSGSGSGTDFTLTISSLQPEDLADYYC

SEQ ID NO: 46 - protein, 10 aa, Artificial Sequence
  Synthetic artificial sequence-FR-L4 amino acid sequence of 6F7L2 skeleton region
FGGGTKLEIK

SEQ ID NO: 47 - protein, 25 aa, Artificial Sequence
  Synthetic artificial sequence-FR-H1 amino acid sequence of 6F7H3 skeleton region
QVQLVQSGAEVVKPGASVKVSCKAS

SEQ ID NO: 48 - protein, 17 aa, Artificial Sequence
  Synthetic artificial sequence-FR-H2 amino acid sequence of 6F7H3 skeleton region
MNWVRQAPGQGLEWIGI

SEQ ID NO: 49 - protein, 38 aa, Artificial Sequence
  Synthetic artificial sequence-FR-H3 amino acid sequence of 6F7H3 skeleton region
SYAQKFQGRVTLTVDKSTSTAYMELSSLRSEDTAVYYC

SEQ ID NO: 50 - protein, 11 aa, Artificial Sequence
  Synthetic artificial sequence-FR-H4 amino acid sequence of 6F7H3 skeleton region
WGAGTTVTVSS

SEQ ID NO: 51 - protein, 26 aa, Artificial Sequence
  Synthetic artificial sequence-FR-L1 amino acid sequence of 6F7L3 skeleton region
NIVMTQSPATLSLSPGERVTLSCRAS

SEQ ID NO: 52 - protein, 17 aa, Artificial Sequence
  Synthetic artificial sequence-FR-L2 amino acid sequence of 6F7L3 skeleton region
LSWYQQKPGQAPRLLIY

SEQ ID NO: 53 - protein, 36 aa, Artificial Sequence
  Synthetic artificial sequence-FR-L3 amino acid sequence of 6F7L3 skeleton region
TRATGIPARFSGSGSGTDFTLTISSLQPEDFAVYYC

SEQ ID NO: 54 - protein, 10 aa, Artificial Sequence
  Synthetic artificial sequence-FR-L4 amino acid sequence of 6F7L3 skeleton region
FGGGTKLEIK

SEQ ID NO: 55 - protein, 330 aa, Artificial Sequence
  Synthetic artificial sequence-Amino acid sequence of the constant region of the heavy chain of IgG1M
ASTKGPSVFPLAPSSKSTSGGTAALGCLVKDYFPEPVTVSWNSGALTSGVHTFPAVLQSSGLYSLSSVVTVPSSSLGTQTYICNVNHKPSNTKVDKKVEPKSCDKTHTCPPCPAPEAAGGPSVFLFPPKPKDTLMISRTPEVTCVVVDVSHEDPEVKFNWYVDGVEVHNAKTKPREEQYNSTYRVVSVLTVLHQDWLNGKEYKCKVSNKALPAPIEKTISKAKGQPREPQVYTLPPSRDELTKNQVSLTCLVKGFYPSDIAVEWESNGQPENNYKTTPPVLDSDGSFFLYSKLTVDKSRWQQGNVFSCSVMHEALHNHYTQKSLSLSPGK

SEQ ID NO: 56 - protein, 327 aa, Artificial Sequence
  Synthetic artificial sequence-Amino acid sequence of the C region of Ig gamma-4 chain in the constant region of heavy chain
ASTKGPSVFPLAPCSRSTSESTAALGCLVKDYFPEPVTVSWNSGALTSGVHTFPAVLQSSGLYSLSSVVTVPSSSLGTKTYTCNVDHKPSNTKVDKRVESKYGPPCPSCPAPEFLGGPSVFLFPPKPKDTLMISRTPEVTCVVVDVSQEDPEVQFNWYVDGVEVHNAKTKPREEQFNSTYRVVSVLTVLHQDWLNGKEYKCKVSNKGLPSSIEKTISKAKGQPREPQVYTLPPSQEEMTKNQVSLTCLVKGFYPSDIAVEWESNGQPENNYKTTPPVLDSDGSFFLYSRLTVDKSRWQEGNVFSCSVMHEALHNHYTQKSLSLSLGK

SEQ ID NO: 57 - protein, 107 aa, Artificial Sequence [sequence omitted]

SEQ ID NO: 58 - protein, 330 aa, Artificial Sequence [sequence omitted]

SEQ ID NO: 59 - protein, 447 aa, Artificial Sequence
  Synthetic artificial sequence- Amino acid sequence of the heavy chain of 6F7H1L1(G1M)
QVQLVQSGAEVVKPGASVKLSCKASGYTFTSYWMNWVRQRPGQGLEWIGMIDPSDSETHNAQKFQGKATLTVDKSTSTAYMHLSSLRSEDTAVYYCARLYRWYFDVWGAGTTVTVSSASTKGPSVFPLAPSSKSTSGGTAALGCLVKDYFPEPVTVSWNSGALTSGVHTFPAVLQSSGLYSLSSVVTVPSSSLGTQTYICNVNHKPSNTKVDKKVEPKSCDKTHTCPPCPAPEAAGGPSVFLFPPKPKDTLMISRTPEVTCVVVDVSHEDPEVKFNWYVDGVEVHNAKTKPREEQYNSTYRVVSVLTVLHQDWLNGKEYKCKVSNKALPAPIEKTISKAKGQPREPQVYTLPPSRDELTKNQVSLTCLVKGFYPSDIAVEWESNGQPENNYKTTPPVLDSDGSFFLYSKLTVDKSRWQQGNVFSCSVMHEALHNHYTQKSLSLSPGK

SEQ ID NO: 60 - protein, 214 aa, Artificial Sequence
  Synthetic artificial sequence- Amino acid sequence of the light chain of 6F7H1L1(G1M)
NIVMTQSPATMSMSPGERVTLSCRASEIVGTYVSWFQQKPGQAPRLLIYGASNRYTGVPARFSGSGSGTDFTLTISSVQPEDLADYHCGQSYNFPYTFGGGTKLEIKRTVAAPSVFIFPPSDEQLKSGTASVVCLLNNFYPREAKVQWKVDNALQSGNSQESVTEQDSKDSTYSLSSTLTLSKADYEKHKVYACEVTHQGLSSPVTKSFNRGEC

SEQ ID NO: 61 - protein, 447 aa, Artificial Sequence
  Synthetic artificial sequence-Amino acid sequence of the heavy chain of 6F7H2L2(G1M)
QVQLVQSGAEVVKPGASVKVSCKASGYTFTSYWMNWVRQRPGQGLEWIGIIDPSDSETSNAQKFQGRVTLTVDKSTSTAYMHLSSLRSEDTAVYYCARLYRWYFDVWGAGTTVTVSSASTKGPSVFPLAPSSKSTSGGTAALGCLVKDYFPEPVTVSWNSGALTSGVHTFPAVLQSSGLYSLSSVVTVPSSSLGTQTYICNVNHKPSNTKVDKKVEPKSCDKTHTCPPCPAPEAAGGPSVFLFPPKPKDTLMISRTPEVTCVVVDVSHEDPEVKFNWYVDGVEVHNAKTKPREEQYNSTYRVVSVLTVLHQDWLNGKEYKCKVSNKALPAPIEKTISKAKGQPREPQVYTLPPSRDELTKNQVSLTCLVKGFYPSDIAVEWESNGQPENNYKTTPPVLDSDGSFFLYSKLTVDKSRWQQGNVFSCSVMHEALHNHYTQKSLSLSPGK

SEQ ID NO: 62 - protein, 214 aa, Artificial Sequence
  Synthetic artificial sequence-Amino acid sequence of the light chain of 6F7H2L2(G1M)
NIVMTQSPATLSLSPGERVTLSCRASEIVGTYVSWFQQKPGQAPRLLIYGASNRATGIPARFSGSGSGTDFTLTISSLQPEDLADYYCGQSYNFPYTFGGGTKLEIKRTVAAPSVFIFPPSDEQLKSGTASVVCLLNNFYPREAKVQWKVDNALQSGNSQESVTEQDSKDSTYSLSSTLTLSKADYEKHKVYACEVTHQGLSSPVTKSFNRGEC

SEQ ID NO: 63 - protein, 447 aa, Artificial Sequence
  Synthetic artificial sequence-Amino acid sequence of the heavy chain of 6F7H3L3(G1M)
QVQLVQSGAEVVKPGASVKVSCKASGYTFTSYWMNWVRQAPGQGLEWIGIIDPSDSETSYAQKFQGRVTLTVDKSTSTAYMELSSLRSEDTAVYYCARLYRWYFDVWGAGTTVTVSSASTKGPSVFPLAPSSKSTSGGTAALGCLVKDYFPEPVTVSWNSGALTSGVHTFPAVLQSSGLYSLSSVVTVPSSSLGTQTYICNVNHKPSNTKVDKKVEPKSCDKTHTCPPCPAPEAAGGPSVFLFPPKPKDTLMISRTPEVTCVVVDVSHEDPEVKFNWYVDGVEVHNAKTKPREEQYNSTYRVVSVLTVLHQDWLNGKEYKCKVSNKALPAPIEKTISKAKGQPREPQVYTLPPSRDELTKNQVSLTCLVKGFYPSDIAVEWESNGQPENNYKTTPPVLDSDGSFFLYSKLTVDKSRWQQGNVFSCSVMHEALHNHYTQKSLSLSPGK

SEQ ID NO: 64 - protein, 214 aa, Artificial Sequence
  Synthetic artificial sequence-Amino acid sequence of the light chain of 6F7H3L3(G1M)
NIVMTQSPATLSLSPGERVTLSCRASEIVGTYLSWYQQKPGQAPRLLIYGASTRATGIPARFSGSGSGTDFTLTISSLQPEDFAVYYCGQSYNFPYTFGGGTKLEIKRTVAAPSVFIFPPSDEQLKSGTASVVCLLNNFYPREAKVQWKVDNALQSGNSQESVTEQDSKDSTYSLSSTLTLSKADYEKHKVYACEVTHQGLSSPVTKSFNRGEC

SEQ ID NO: 65 - protein, 444 aa, Artificial Sequence
  Synthetic artificial sequence-Amino acid sequence of the heavy chain of 6F7H1L1(hG4)
QVQLVQSGAEVVKPGASVKLSCKASGYTFTSYWMNWVRQRPGQGLEWIGMIDPSDSETHNAQKFQGKATLTVDKSTSTAYMHLSSLRSEDTAVYYCARLYRWYFDVWGAGTTVTVSSASTKGPSVFPLAPCSRSTSESTAALGCLVKDYFPEPVTVSWNSGALTSGVHTFPAVLQSSGLYSLSSVVTVPSSSLGTKTYTCNVDHKPSNTKVDKRVESKYGPPCPSCPAPEFLGGPSVFLFPPKPKDTLMISRTPEVTCVVVDVSQEDPEVQFNWYVDGVEVHNAKTKPREEQFNSTYRVVSVLTVLHQDWLNGKEYKCKVSNKGLPSSIEKTISKAKGQPREPQVYTLPPSQEEMTKNQVSLTCLVKGFYPSDIAVEWESNGQPENNYKTTPPVLDSDGSFFLYSRLTVDKSRWQEGNVFSCSVMHEALHNHYTQKSLSLSLGK

SEQ ID NO: 66 - protein, 214 aa, Artificial Sequence; identical to SEQ ID NO: 60
  Synthetic artificial sequence-Amino acid sequence of the light chain of 6F7H1L1(hG4)

SEQ ID NO: 67 - protein, 444 aa, Artificial Sequence
  Synthetic artificial sequence-Amino acid sequence of the heavy chain of 6F7H2L2(hG4)
QVQLVQSGAEVVKPGASVKVSCKASGYTFTSYWMNWVRQRPGQGLEWIGIIDPSDSETSNAQKFQGRVTLTVDKSTSTAYMHLSSLRSEDTAVYYCARLYRWYFDVWGAGTTVTVSSASTKGPSVFPLAPCSRSTSESTAALGCLVKDYFPEPVTVSWNSGALTSGVHTFPAVLQSSGLYSLSSVVTVPSSSLGTKTYTCNVDHKPSNTKVDKRVESKYGPPCPSCPAPEFLGGPSVFLFPPKPKDTLMISRTPEVTCVVVDVSQEDPEVQFNWYVDGVEVHNAKTKPREEQFNSTYRVVSVLTVLHQDWLNGKEYKCKVSNKGLPSSIEKTISKAKGQPREPQVYTLPPSQEEMTKNQVSLTCLVKGFYPSDIAVEWESNGQPENNYKTTPPVLDSDGSFFLYSRLTVDKSRWQEGNVFSCSVMHEALHNHYTQKSLSLSLGK

SEQ ID NO: 68 - protein, 214 aa, Artificial Sequence; identical to SEQ ID NO: 62
  Synthetic artificial sequence-Amino acid sequence of the light chain of 6F7H2L2(hG4)

SEQ ID NO: 69 - protein, 444 aa, Artificial Sequence
  Synthetic artificial sequence-Amino acid sequence of the heavy chain of 6F7H3L3(hG4)
QVQLVQSGAEVVKPGASVKVSCKASGYTFTSYWMNWVRQAPGQGLEWIGIIDPSDSETSYAQKFQGRVTLTVDKSTSTAYMELSSLRSEDTAVYYCARLYRWYFDVWGAGTTVTVSSASTKGPSVFPLAPCSRSTSESTAALGCLVKDYFPEPVTVSWNSGALTSGVHTFPAVLQSSGLYSLSSVVTVPSSSLGTKTYTCNVDHKPSNTKVDKRVESKYGPPCPSCPAPEFLGGPSVFLFPPKPKDTLMISRTPEVTCVVVDVSQEDPEVQFNWYVDGVEVHNAKTKPREEQFNSTYRVVSVLTVLHQDWLNGKEYKCKVSNKGLPSSIEKTISKAKGQPREPQVYTLPPSQEEMTKNQVSLTCLVKGFYPSDIAVEWESNGQPENNYKTTPPVLDSDGSFFLYSRLTVDKSRWQEGNVFSCSVMHEALHNHYTQKSLSLSLGK

SEQ ID NO: 70 - protein, 214 aa, Artificial Sequence; identical to SEQ ID NO: 64
  Synthetic artificial sequence-Amino acid sequence of the light chain of 6F7H3L3(hG4)

SEQ ID NO: 71 - protein, 232 aa, Artificial Sequence
  Synthetic artificial sequence-Sequence of mFc tags
PRGPTIKPCPPCKCPAPNLLGGPSVFIFPPKIKDVLMISLSPIVTCVVVDVSEDDPDVQISWFVNNVEVHTAQTQTHREDYNSTLRVVSALPIQHQDWMSGKEFKCKVNNKDLPAPIERTISKPKGSVRAPQVYVLPPPEEEMTKKQVTLTCMVTDFMPEDIYVEWTNNGKTELNYKNTEPVLDSDGSYFMYSKLRVEKKNWVERNSYSCSVVHEGLHNHHTTKSFSRTPGK

SEQ ID NO: 72 - protein, 443 aa, Artificial Sequence
  Synthetic artificial sequence-The heavy chain sequence of hIgG
EVQLEQSGAELMKPGASVKISCKATGYTFTTYWIEWIKQRPGHSLEWIGEILPGSDSTYYNEKVKGKVTFTADASSNTAYMQLSSLTSEDSAVYYCARGDGFYVYWGQGTTLTVSSASTKGPSVFPLAPCSRSTSESTAALGCLVKDYFPEPVTVSWNSGALTSGVHTFPAVLQSSGLYSLSSVVTVPSSSLGTKTYTCNVDHKPSNTKVDKRVESKYGPPCPPCPAPEFLGGPSVFLFPPKPKDTLMISRTPEVTCVVVDVSQEDPEVQFNWYVDGVEVHNAKTKPREEQFNSTYRVVSVLTVLHQDWLNGKEYKCKVSNKGLPSSIEKTISKAKGQPREPQVYTLPPSQEEMTKNQVSLTCLVKGFYPSDIAVEWESNGQPENNYKTTPPVLDSDGSFFLYSRLTVDKSRWQEGNVFSCSVMHEALHNHYTQKSLSLSLGK

SEQ ID NO: 73 - protein, 214 aa, Artificial Sequence
  Synthetic artificial sequence-Light chain sequence of hIgG
DIELTQSPATLSVTPGDSVSLSCRASQSISNNLHWYQQKSHESPRLLIKYTSQSMSGIPSRFSGSGSGTDFTLSINSVETEDFGVYFCQQSGSWPRTFGGGTKLDIKRTVAAPSVFIFPPSDEQLKSGTASVVCLLNNFYPREAKVQWKVDNALQSGNSQESVTEQDSKDSTYSLSSTLTLSKADYEKHKVYACEVTHQGLSSPVTKSFNRGEC

SEQ ID NO: 74 - protein, 7 aa, Artificial Sequence
  Synthetic artificial sequence-TEV amino acid sequence
ENLYFQG

SEQ ID NO: 75 - protein, 116 aa, Artificial Sequence
  Synthetic artificial sequence-Heavy chain variable region sequence of hIgG
EVQLEQSGAELMKPGASVKISCKATGYTFTTYWIEWIKQRPGHSLEWIGEILPGSDSTYYNEKVKGKVTFTADASSNTAYMQLSSLTSEDSAVYYCARGDGFYVYWGQGTTLTVSS

SEQ ID NO: 76 - protein, 107 aa, Artificial Sequence
  Synthetic artificial sequence-Light chain variable region sequence of hIgG
DIELTQSPATLSVTPGDSVSLSCRASQSISNNLHWYQQKSHESPRLLIKYTSQSMSGIPSRFSGSGSGTDFTLSINSVETEDFGVYFCQQSGSWPRTFGGGTKLDIK

SEQ ID NO: 77 - DNA, 2139 bp, Artificial Sequence
  Synthetic artificial sequence- Nucleic acid sequence of CP004(hG1TM) heavy chain
gaagtgcagctggtcgagtctgggggagggctggtgcagcccggcgggtcactgcgactgagctgcgcagcttccggattcgcctttagctcctacgacatgtcctgggtgcgacaggcaccaggaaagggactggattgggtcgctactatctcaggaggcgggagatacacctactatcctgacagcgtcaagggccggttcacaatctctagagataacagtaagaacaatctgtatctgcagatgaacagcctgagggctgaggacaccgcactgtactattgtgccaaccgctacggggaagcatggtttgcctattgggggcagggaaccctggtgacagtctctagtgccagcaccaaagggcccagcgtgtttcctctcgccccctcctccaaaagcaccagcggaggaaccgctgctctcggatgtctggtgaaggactacttccctgaacccgtcaccgtgagctggaatagcggcgctctgacaagcggagtccatacattccctgctgtgctgcaaagcagcggactctattccctgtccagcgtcgtcacagtgcccagcagcagcctgggcacccagacctacatctgtaacgtcaaccacaagccctccaacaccaaggtggacaagaaagtggagcccaaatcctgcgacaagacacacacctgtcccccctgtcctgctcccgaagctgctggagcccctagcgtcttcctctttcctcccaaacccaaggacaccctcatgatcagcagaacccctgaagtcacctgtgtcgtcgtggatgtcagccatgaggaccccgaggtgaaattcaactggtatgtcgatggcgtcgaggtgcacaacgccaaaaccaagcccagggaggaacagtacaactccacctacagggtggtgtccgtgctgacagtcctccaccaggactggctgaacggcaaggagtacaagtgcaaggtgtccaacaaggctctccctgcccccattgagaagaccatcagcaaggccaaaggccaacccagggagccccaggtctatacactgcctccctccagggacgaactcaccaagaaccaggtgtccctgacctgcctggtcaagggcttttatcccagcgacatcgccgtcgagtgggagtccaacggacagcccgagaataactacaagaccacccctcctgtcctcgactccgacggctccttcttcctgtacagcaaactgaccgtggataagtccagatggcagcagggcaatgtcttttcatgttccgtgatgcacgaggcactgcacaaccactatacccagaagtctctgagtctgtcaccaggaaaaggaggaggaggctctggaggaggcggaagtggaggcggaggatcaggagggggaggatctcaggtgcagctggtcgaatccggagccgaggtgaagaaacccggcgcttccgtgaaggtctcttgcaaagcatcaggctacagcttcacagggtatactatgaactgggtgcggcaggcacctggacagtgtctggaatggatcggcctgattaacccatacaacaacatcactaactacgcccagaagttccagggccgggtgacttttaccgtggacactagcatttccaccgcttacatggagctgagtcggctgagatcagacgataccggcgtgtatttttgcgcaaggctggattacagaagttattggggacagggaacacttgttacagtctctgctggaggaggcggatctggaggaggaggatctggcggaggaggcagtggaggaggaggatcacaggctgtggttactcaggaaccaagcctgaccgtgagccccggaggcacagtcactctgacctgtgggagctccacaggagctgtgaccacatctaacttccctaattgggtgcagcagaagccaggacaggcacctcgatccctgatcgggggaaccaacaacaaggccagctggacacccgccagattttctggcagtctgctgggcgggaaagccgctctgaccattagcggcgctcagcctgaggacgaagcagagtactattgcgccctgtggtatagtaatcattgggtgttcgggtgtgggacaaaactgaccgtgctgaga

SEQ ID NO: 78 - protein, 713 aa, Artificial Sequence
  Synthetic artificial sequence- Amino acid sequence of the heavy chain of CP004(hG1TM)
EVQLVESGGGLVQPGGSLRLSCAASGFAFSSYDMSWVRQAPGKGLDWVATISGGGRYTYYPDSVKGRFTISRDNSKNNLYLQMNSLRAEDTALYYCANRYGEAWFAYWGQGTLVTVSSASTKGPSVFPLAPSSKSTSGGTAALGCLVKDYFPEPVTVSWNSGALTSGVHTFPAVLQSSGLYSLSSVVTVPSSSLGTQTYICNVNHKPSNTKVDKKVEPKSCDKTHTCPPCPAPEAAGAPSVFLFPPKPKDTLMISRTPEVTCVVVDVSHEDPEVKFNWYVDGVEVHNAKTKPREEQYNSTYRVVSVLTVLHQDWLNGKEYKCKVSNKALPAPIEKTISKAKGQPREPQVYTLPPSRDELTKNQVSLTCLVKGFYPSDIAVEWESNGQPENNYKTTPPVLDSDGSFFLYSKLTVDKSRWQQGNVFSCSVMHEALHNHYTQKSLSLSPGKGGGGSGGGGSGGGGSGGGGSQVQLVESGAEVKKPGASVKVSCKASGYSFTGYTMNWVRQAPGQCLEWIGLINPYNNITNYAQKFQGRVTFTVDTSISTAYMELSRLRSDDTGVYFCARLDYRSYWGQGTLVTVSAGGGGSGGGGSGGGGSGGGGSQAVVTQEPSLTVSPGGTVTLTCGSSTGAVTTSNFPNWVQQKPGQAPRSLIGGTNNKASWTPARFSGSLLGGKAALTISGAQPEDEAEYYCALWYSNHWVFGCGTKLTVLR

SEQ ID NO: 79 - DNA, 642 bp, Artificial Sequence
  Synthetic artificial sequence-Nucleic acid sequence of the light chain of CP004(hG1TM)
gacattcagatgactcagagcccctcctccatgtccgcctctgtgggcgacagggtcaccttcacatgccgcgctagtcaggatatcaacacctacctgagctggtttcagcagaagccagggaaaagccccaagacactgatctaccgggctaatagactggtgtctggagtcccaagtcggttcagtggctcagggagcggacaggactacactctgaccatcagctccctgcagcctgaggacatggcaacctactattgcctgcagtatgatgagttcccactgacctttggcgccgggacaaaactggagctgaagcgaactgtggccgctccctccgtcttcatttttcccccttctgacgaacagctgaaatcaggcacagccagcgtggtctgtctgctgaacaatttctaccctagagaggcaaaagtgcagtggaaggtcgataacgccctgcagtccggcaacagccaggagagtgtgactgaacaggactcaaaagatagcacctattccctgtctagtacactgactctgtccaaggctgattacgagaagcacaaagtgtatgcatgcgaagtgacacatcagggactgtcaagccccgtgactaagtcttttaaccggggcgaatgt

SEQ ID NO: 80 - protein, 214 aa, Artificial Sequence
  Synthetic artificial sequence- Amino acid sequence of the light chain of CP004(hG1TM)
DIQMTQSPSSMSASVGDRVTFTCRASQDINTYLSWFQQKPGKSPKTLIYRANRLVSGVPSRFSGSGSGQDYTLTISSLQPEDMATYYCLQYDEFPLTFGAGTKLELKRTVAAPSVFIFPPSDEQLKSGTASVVCLLNNFYPREAKVQWKVDNALQSGNSQESVTEQDSKDSTYSLSSTLTLSKADYEKHKVYACEVTHQGLSSPVTKSFNRGEC

SEQ ID NO: 81 - DNA, 1344 bp, Artificial Sequence
  Synthetic artificial sequence-Nucleic acid sequence of Penpulimab heavy chain
gaagtgcagctggtcgagtctgggggagggctggtgcagcccggcgggtcactgcgactgagctgcgcagcttccggattcgcctttagctcctacgacatgtcctgggtgcgacaggcaccaggaaagggactggattgggtcgctactatctcaggaggcgggagatacacctactatcctgacagcgtcaagggccggttcacaatctctagagataacagtaagaacaatctgtatctgcagatgaacagcctgagggctgaggacaccgcactgtactattgtgccaaccgctacggggaagcatggtttgcctattgggggcagggaaccctggtgacagtctctagtgccagcaccaaagggcccagcgtgtttcctctcgccccctcctccaaaagcaccagcggaggaaccgctgctctcggatgtctggtgaaggactacttccctgaacccgtcaccgtgagctggaatagcggcgctctgacaagcggagtccatacattccctgctgtgctgcaaagcagcggactctattccctgtccagcgtcgtcacagtgcccagcagcagcctgggcacccagacctacatctgtaacgtcaaccacaagccctccaacaccaaggtggacaagaaagtggagcccaaatcctgcgacaagacacacacctgtcccccctgtcctgctcccgaagctgctggagcccctagcgtcttcctctttcctcccaaacccaaggacaccctcatgatcagcagaacccctgaagtcacctgtgtcgtcgtggatgtcagccatgaggaccccgaggtgaaattcaactggtatgtcgatggcgtcgaggtgcacaacgccaaaaccaagcccagggaggaacagtacaactccacctacagggtggtgtccgtgctgacagtcctccaccaggactggctgaacggcaaggagtacaagtgcaaggtgtccaacaaggctctccctgcccccattgagaagaccatcagcaaggccaaaggccaacccagggagccccaggtctatacactgcctccctccagggacgaactcaccaagaaccaggtgtccctgacctgcctggtcaagggcttttatcccagcgacatcgccgtcgagtgggagtccaacggacagcccgagaataactacaagaccacccctcctgtcctcgactccgacggctccttcttcctgtacagcaagctgaccgtggacaaaagcaggtggcagcagggaaacgtgttctcctgcagcgtgatgcacgaagccctccacaaccactacacccagaaaagcctgtccctgagccccggcaaa

SEQ ID NO: 82 - protein, 448 aa, Artificial Sequence
  Synthetic artificial sequence-Amino acid sequence of the heavy chain of Penpulimab
EVQLVESGGGLVQPGGSLRLSCAASGFAFSSYDMSWVRQAPGKGLDWVATISGGGRYTYYPDSVKGRFTISRDNSKNNLYLQMNSLRAEDTALYYCANRYGEAWFAYWGQGTLVTVSSASTKGPSVFPLAPSSKSTSGGTAALGCLVKDYFPEPVTVSWNSGALTSGVHTFPAVLQSSGLYSLSSVVTVPSSSLGTQTYICNVNHKPSNTKVDKKVEPKSCDKTHTCPPCPAPEAAGAPSVFLFPPKPKDTLMISRTPEVTCVVVDVSHEDPEVKFNWYVDGVEVHNAKTKPREEQYNSTYRVVSVLTVLHQDWLNGKEYKCKVSNKALPAPIEKTISKAKGQPREPQVYTLPPSRDELTKNQVSLTCLVKGFYPSDIAVEWESNGQPENNYKTTPPVLDSDGSFFLYSKLTVDKSRWQQGNVFSCSVMHEALHNHYTQKSLSLSPGK

SEQ ID NO: 83 - DNA, 642 bp, Artificial Sequence; identical to SEQ ID NO: 79
  Synthetic artificial sequence-Nucleic acid sequence of the light chain of Penpulimab

SEQ ID NO: 84 - protein, 214 aa, Artificial Sequence; identical to SEQ ID NO: 80
  Synthetic artificial sequence-Amino acid sequence of the light chain of Penpulimab

SEQ ID NO: 85 - protein, 444 aa, Artificial Sequence
  Synthetic artificial sequence-Amino acid sequence of Hu5F9-G4 heavy chain
QVQLVQSGAEVKKPGASVKVSCKASGYTFTNYNMHWVRQAPGQRLEWMGTIYPGNDDTSYNQKFKDRVTITADTSASTAYMELSSLRSEDTAVYYCARGGYRAMDYWGQGTLVTVSSASTKGPSVFPLAPCSRSTSESTAALGCLVKDYFPEPVTVSWNSGALTSGVHTFPAVLQSSGLYSLSSVVTVPSSSLGTKTYTCNVDHKPSNTKVDKRVESKYGPPCPPCPAPEFLGGPSVFLFPPKPKDTLMISRTPEVTCVVVDVSQEDPEVQFNWYVDGVEVHNAKTKPREEQFNSTYRVVSVLTVLHQDWLNGKEYKCKVSNKGLPSSIEKTISKAKGQPREPQVYTLPPSQEEMTKNQVSLTCLVKGFYPSDIAVEWESNGQPENNYKTTPPVLDSDGSFFLYSRLTVDKSRWQEGNVFSCSVMHEALHNHYTQKSLSLSLGK

SEQ ID NO: 86 - protein, 219 aa, Artificial Sequence
  Synthetic artificial sequence-Amino acid sequence of Hu5F9-G4 light chain
DIVMTQSPLSLPVTPGEPASISCRSSQSIVYSNGNTYLGWYLQKPGQSPQLLIYKVSNRFSGVPDRFSGSGSGTDFTLKISRVEAEDVGVYYCFQGSHVPYTFGQGTKLEIKRTVAAPSVFIFPPSDEQLKSGTASVVCLLNNFYPREAKVQWKVDNALQSGNSQESVTEQDSKDSTYSLSSTLTLSKADYEKHKVYACEVTHQGLSSPVTKSFNRGEC

SEQ ID NO: 87 - protein, 118 aa, Artificial Sequence
  Synthetic artificial sequence- Amino acid sequence of the heavy chain variable region of 14C12
EVKLVESGGGLVKPGGSLKLSCAASGFAFSSYDMSWVRQTPEKRLEWVATISGGGRYTYYPDSVKGRFTISRDNARNTLYLQMSSLRSEDTALYYCANRYGEAWFAYWGQGTLVTVSA

SEQ ID NO: 88 - protein, 107 aa, Artificial Sequence
  Synthetic artificial sequence-Amino acid sequence of the variable region of the light chain of 14C12
DIKMTQSPSSMYASLGERVTFTCKASQDINTYLSWFQQKPGKSPKTLIYRANRLVDGVPSRFSGSGSGQDYSLTISSLEYEDMGIYYCLQYDEFPLTFGAGTKLELK

SEQ ID NO: 89 - protein, 8 aa, Artificial Sequence
  Synthetic artificial sequence-Amino acid sequence of HCDR1 of 14C12
GFAFSSYD

SEQ ID NO: 90 - protein, 8 aa, Artificial Sequence
  Synthetic artificial sequence-Amino acid sequence of HCDR2 of 14C12
ISGGGRYT

SEQ ID NO: 91 - protein, 11 aa, Artificial Sequence
  Synthetic artificial sequence-Amino acid sequence of HCDR3 of 14C12
ANRYGEAWFAY

SEQ ID NO: 92 - protein, 6 aa, Artificial Sequence
  Synthetic artificial sequence-Amino acid sequence of LCDR1 of 14C12
QDINTY

SEQ ID NO: 93 - protein, 3 aa, Artificial Sequence
  Synthetic artificial sequence-Amino acid sequence of LCDR2 of 14C12
RAN

SEQ ID NO: 94 - protein, 9 aa, Artificial Sequence
  Synthetic artificial sequence-Amino acid sequence of LCDR3 of 14C12
LQYDEFPLT

SEQ ID NO: 95 - protein, 124 aa, Artificial Sequence
  Synthetic artificial sequence-Amino acid sequence of the heavy chain variable region of 4G10
QVKLQESGPELVKPGASMKISCKASGYSFTGYTMNWVKQSHGKNLEWIGLINPYNNITNYNQKFMGKATFTVDKSSSTAYMELLRLTSEDSGVYFCARLDYRSYWGQGTLVTVSAAKTTPPSVY

SEQ ID NO: 96 - protein, 126 aa, Artificial Sequence
  Synthetic artificial sequence-Amino acid sequence of the variable region of the light chain of 4G10
QAVVTQESALTTSPGETVTLTCRSSTGAVTTSNFANWVQEKPDHLFTSLIGGTNNRAPGVPARFSGSLIGDKAALTITGAQTEDEAIYFCALWYSNHWVFGGGTKLTVLGQPKSSPSVTLFQGQFC

SEQ ID NO: 97 - protein, 8 aa, Artificial Sequence
  Synthetic artificial sequence-Amino acid sequence of HCDR1 of 4G10
GYSFTGYT

SEQ ID NO: 98 - protein, 8 aa, Artificial Sequence
  Synthetic artificial sequence-Amino acid sequence of HCDR2 of 4G10
INPYNNIT

SEQ ID NO: 99 - protein, 8 aa, Artificial Sequence
  Synthetic artificial sequence- Amino acid sequence of HCDR3 of 4G10
ARLDYRSY

SEQ ID NO: 100 - protein, 9 aa, Artificial Sequence
  Synthetic artificial sequence-Amino acid sequence of LCDR1 of 4G10
TGAVTTSNF

SEQ ID NO: 101 - protein, 3 aa, Artificial Sequence
  Synthetic artificial sequence-Amino acid sequence of LCDR2 of 4G10
GTN

SEQ ID NO: 102 - protein, 9 aa, Artificial Sequence
  Synthetic artificial sequence-Amino acid sequence of LCDR3 of 4G10
ALWYSNHWV

SEQ ID NO: 103 - protein, 118 aa, Artificial Sequence
  Synthetic artificial sequence-Amino acid sequence of the heavy chain variable region of humanized monoclonal antibody 14C12H1L1
EVQLVESGGGLVQPGGSLRLSCAASGFAFSSYDMSWVRQAPGKGLDWVATISGGGRYTYYPDSVKGRFTISRDNSKNNLYLQMNSLRAEDTALYYCANRYGEAWFAYWGQGTLVTVSS

SEQ ID NO: 104 - protein, 108 aa, Artificial Sequence
  Synthetic artificial sequence-Amino acid sequence of the variable region of the light chain of humanized monoclonal antibody 14C12H1L1(M)
DIQMTQSPSSMSASVGDRVTFTCRASQDINTYLSWFQQKPGKSPKTLIYRANRLVSGVPSRFSGSGSGQDYTLTISSLQPEDMATYYCLQYDEFPLTFGAGTKLELKR

SEQ ID NO: 105 - protein, 8 aa, Artificial Sequence
  Synthetic artificial sequence-Amino acid sequence of HCDR1 in variable region of 14C12H1L1(M) heavy chain
GFAFSSYD

SEQ ID NO: 106 - protein, 8 aa, Artificial Sequence
  Synthetic artificial sequence-Amino acid sequence of HCDR2 in variable region of 14C12H1L1(M) heavy chain
ISGGGRYT

SEQ ID NO: 107 - protein, 11 aa, Artificial Sequence
  Synthetic artificial sequence-Amino acid sequence of HCDR3 in variable region of 14C12H1L1(M) heavy chain
ANRYGEAWFAY

SEQ ID NO: 108 - protein, 6 aa, Artificial Sequence
  Synthetic artificial sequence-Amino acid sequence of LCDR1 in variable region of 14C12H1L1(M) light chain
QDINTY

SEQ ID NO: 109 - protein, 3 aa, Artificial Sequence
  Synthetic artificial sequence-Amino acid sequence of LCDR2 in variable region of 14C12H1L1(M) light chain
RAN

SEQ ID NO: 110 - protein, 9 aa, Artificial Sequence
  Synthetic artificial sequence-Amino acid sequence of LCDR3 in variable region of 14C12H1L1(M) light chain
LQYDEFPLT

SEQ ID NO: 111 - protein, 123 aa, Artificial Sequence [sequence omitted]

SEQ ID NO: 112 - protein, 107 aa, Artificial Sequence [sequence omitted]

SEQ ID NO: 113 - protein, 8 aa, Artificial Sequence
  Synthetic artificial sequence-Amino acid sequence of HCDR1 in the heavy chain variable region of Bevacizumab
GYTFTNYG

SEQ ID NO: 114 - protein, 8 aa, Artificial Sequence
  Synthetic artificial sequence-Amino acid sequence of HCDR2 in the heavy chain variable region of Bevacizumab
INTYTGEP

SEQ ID NO: 115 - protein, 16 aa, Artificial Sequence
  Synthetic artificial sequence-Amino acid sequence of HCDR3 in the heavy chain variable region of Bevacizumab
AKYPHYYGSSHWYFDV

SEQ ID NO: 116 - protein, 6 aa, Artificial Sequence
  Synthetic artificial sequence-Amino acid sequence of LCDR1 in the variable region of the light chain of Bevacizumab
QDISNY

SEQ ID NO: 117 - protein, 3 aa, Artificial Sequence
  Synthetic artificial sequence-Amino acid sequence of LCDR2 in the variable region of the light chain of Bevacizumab
FTS

SEQ ID NO: 118 - protein, 9 aa, Artificial Sequence
  Synthetic artificial sequence-Amino acid sequence of LCDR3 in the variable region of the light chain of Bevacizumab
QQYSTVPWT

SEQ ID NO: 119 - protein, 15 aa, Artificial Sequence
  Synthetic artificial sequence-Amino acid sequence of connector 1
GGGGSGGGGSGGGGS

SEQ ID NO: 120 - protein, 20 aa, Artificial Sequence
  Synthetic artificial sequence-Amino acid sequence of connector 2
GGGGSGGGGSGGGGSGGGGS

SEQ ID NO: 121 - protein, 118 aa, Artificial Sequence; identical to SEQ ID NO: 103
  Synthetic artificial sequence-Amino acid sequence of the heavy chain variable region of Penpulimab

SEQ ID NO: 122 - protein, 107 aa, Artificial Sequence
  Synthetic artificial sequence-Amino acid sequence of the variable region of the light chain of Penpulimab
DIQMTQSPSSMSASVGDRVTFTCRASQDINTYLSWFQQKPGKSPKTLIYRANRLVSGVPSRFSGSGSGQDYTLTISSLQPEDMATYYCLQYDEFPLTFGAGTKLELK

SEQ ID NO: 123 - protein, 8 aa, Artificial Sequence
  Synthetic artificial sequence-Amino acid sequence of HCDR1 of Penpulimab
GFAFSSYD

SEQ ID NO: 124 - protein, 8 aa, Artificial Sequence
  Synthetic artificial sequence-Amino acid sequence of HCDR2 of Penpulimab
ISGGGRYT

SEQ ID NO: 125 - protein, 11 aa, Artificial Sequence
  Synthetic artificial sequence-Amino acid sequence of HCDR3 of Penpulimab
ANRYGEAWFAY

SEQ ID NO: 126 - protein, 6 aa, Artificial Sequence
  Synthetic artificial sequence-Amino acid sequence of LCDR1 of Penpulimab
QDINTY

SEQ ID NO: 127 - protein, 3 aa, Artificial Sequence
  Synthetic artificial sequence-Amino acid sequence of LCDR2 of Penpulimab
RAN

SEQ ID NO: 128 - protein, 9 aa, Artificial Sequence
  Synthetic artificial sequence-Amino acid sequence of LCDR3 of Penpulimab
LQYDEFPLT

SEQ ID NO: 129 - protein, 118 aa, Artificial Sequence; identical to SEQ ID NO: 103
  Synthetic artificial sequence-Amino acid sequence of the heavy chain variable region of 14C12H1L1

SEQ ID NO: 130 - protein, 107 aa, Artificial Sequence; identical to SEQ ID NO: 122
  Synthetic artificial sequence-Amino acid sequence of the variable region of the light chain of 14C12H1L1

SEQ ID NO: 131 - protein, 115 aa, Artificial Sequence
  Synthetic artificial sequence- Amino acid sequence of the heavy chain variable region of 4G10H1L1
QVQLVESGAELVKPGASMKISCKASGYSFTGYTMNWVKQAPGQGLEWIGLINPYNNITNYNQKFMGKATFTVDKSISTAYMELSRLTSDDSGVYFCARLDYRSYWGQGTLVTVSA

SEQ ID NO: 132 - protein, 109 aa, Artificial Sequence
  Synthetic artificial sequence-Amino acid sequence of the variable region of the light chain of 4G10H1L1
QAVVTQEPSLTVSPGGTVTLTCGSSTGAVTTSNFANWVQEKPGQAFRSLIGGTNNRASWVPARFSGSLLGGKAALTISGAQPEDEAEYFCALWYSNHWVFGGGTKLTVL

SEQ ID NO: 133 - protein, 115 aa, Artificial Sequence
  Synthetic artificial sequence-Amino acid sequence of the heavy chain variable region of 4G10H3L3
QVQLVESGAEVKKPGASVKVSCKASGYSFTGYTMNWVRQAPGQGLEWIGLINPYNNITNYAQKFQGRVTFTVDTSISTAYMELSRLRSDDTGVYFCARLDYRSYWGQGTLVTVSA

SEQ ID NO: 134 - protein, 109 aa, Artificial Sequence
  Synthetic artificial sequence-Amino acid sequence of the variable region of the light chain of 4G10H3L3
QAVVTQEPSLTVSPGGTVTLTCGSSTGAVTTSNFPNWVQQKPGQAPRSLIGGTNNKASWTPARFSGSLLGGKAALTISGAQPEDEAEYYCALWYSNHWVFGGGTKLTVL

SEQ ID NO: 135 - protein, 115 aa, Artificial Sequence
  Synthetic artificial sequence-Amino acid sequence of 4G10H1V(M)
QVQLVESGAELVKPGASMKISCKASGYSFTGYTMNWVKQAPGQCLEWIGLINPYNNITNYNQKFMGKATFTVDKSISTAYMELSRLTSDDSGVYFCARLDYRSYWGQGTLVTVSA

SEQ ID NO: 136 - protein, 110 aa, Artificial Sequence
  Synthetic artificial sequence- Amino acid sequence of 4G10L1V(M)
QAVVTQEPSLTVSPGGTVTLTCGSSTGAVTTSNFANWVQEKPGQAFRSLIGGTNNRASWVPARFSGSLLGGKAALTISGAQPEDEAEYFCALWYSNHWVFGCGTKLTVLR

SEQ ID NO: 137 - protein, 115 aa, Artificial Sequence
  Synthetic artificial sequence-Amino acid sequence of 4G10H3V(M)
QVQLVESGAEVKKPGASVKVSCKASGYSFTGYTMNWVRQAPGQCLEWIGLINPYNNITNYAQKFQGRVTFTVDTSISTAYMELSRLRSDDTGVYFCARLDYRSYWGQGTLVTVSA

SEQ ID NO: 138 - protein, 110 aa, Artificial Sequence
  Synthetic artificial sequence-Amino acid sequence of 4G10L3V(M)
QAVVTQEPSLTVSPGGTVTLTCGSSTGAVTTSNFPNWVQQKPGQAPRSLIGGTNNKASWTPARFSGSLLGGKAALTISGAQPEDEAEYYCALWYSNHWVFGCGTKLTVLR

SEQ ID NO: 139 - protein, 448 aa, Artificial Sequence; identical to SEQ ID NO: 82
  Synthetic artificial sequence-Amino acid sequence of the heavy chain of immunoglobulin moiety in CP004(hG1TM)

SEQ ID NO: 140 - protein, 453 aa, Artificial Sequence
  Synthetic artificial sequence-Amino acid sequence of the heavy chain of Bevacizumab
EVQLVESGGGLVQPGGSLRLSCAASGYTFTNYGMNWVRQAPGKGLEWVGWINTYTGEPTYAADFKRRFTFSLDTSKSTAYLQMNSLRAEDTAVYYCAKYPHYYGSSHWYFDVWGQGTLVTVSSASTKGPSVFPLAPSSKSTSGGTAALGCLVKDYFPEPVTVSWNSGALTSGVHTFPAVLQSSGLYSLSSVVTVPSSSLGTQTYICNVNHKPSNTKVDKKVEPKSCDKTHTCPPCPAPELLGGPSVFLFPPKPKDTLMISRTPEVTCVVVDVSHEDPEVKFNWYVDGVEVHNAKTKPREEQYNSTYRVVSVLTVLHQDWLNGKEYKCKVSNKALPAPIEKTISKAKGQPREPQVYTLPPSRDELTKNQVSLTCLVKGFYPSDIAVEWESNGQPENNYKTTPPVLDSDGSFFLYSKLTVDKSRWQQGNVFSCSVMHEALHNHYTQKSLSLSPGK

SEQ ID NO: 141 - protein, 719 aa, Artificial Sequence
  Synthetic artificial sequence-Amino acid sequence of VP101(hG1DM) heavy chain
EVQLVESGGGLVQPGGSLRLSCAASGYTFTNYGMNWVRQAPGKGLEWVGWINTYTGEPTYAADFKRRFTFSLDTSKSTAYLQMNSLRAEDTAVYYCAKYPHYYGSSHWYFDVWGQGTLVTVSSASTKGPSVFPLAPSSKSTSGGTAALGCLVKDYFPEPVTVSWNSGALTSGVHTFPAVLQSSGLYSLSSVVTVPSSSLGTQTYICNVNHKPSNTKVDKKVEPKSCDKTHTCPPCPAPEAAGGPSVFLFPPKPKDTLMISRTPEVTCVVVDVSHEDPEVKFNWYVDGVEVHNAKTKPREEQYNSTYRVVSVLTVLHQDWLNGKEYKCKVSNKALPAPIEKTISKAKGQPREPQVYTLPPSRDELTKNQVSLTCLVKGFYPSDIAVEWESNGQPENNYKTTPPVLDSDGSFFLYSKLTVDKSRWQQGNVFSCSVMHEALHNHYTQKSLSLSPGKGGGGSGGGGSGGGGSGGGGSEVQLVESGGGLVQPGGSLRLSCAASGFAFSSYDMSWVRQAPGKGLDWVATISGGGRYTYYPDSVKGRFTISRDNSKNNLYLQMNSLRAEDTALYYCANRYGEAWFAYWGQGTLVTVSSGGGGSGGGGSGGGGSGGGGSDIQMTQSPSSMSASVGDRVTFTCRASQDINTYLSWFQQKPGKSPKTLIYRANRLVSGVPSRFSGSGSGQDYTLTISSLQPEDMATYYCLQYDEFPLTFGAGTKLELKR

SEQ ID NO: 142 - DNA, 2157 bp, Artificial Sequence
  Synthetic artificial sequence-Nucleic acid sequence of VP101(hG1DM) heavy chain
gaggtgcagctggtcgagtccgggggggggctggtgcagccaggcgggtctctgaggctgagttgcgccgcttcagggtacaccttcacaaactatggaatgaattgggtgcgccaggcaccaggaaagggactggagtgggtcggctggatcaacacttacaccggggaacctacctatgcagccgactttaagcggcggttcaccttcagcctggatacaagcaaatccactgcctacctgcagatgaacagcctgcgagctgaggacaccgcagtctactattgtgctaaatatccccactactatgggagcagccattggtattttgacgtgtgggggcaggggactctggtgacagtgagcagcgcaagcaccaaagggcccagcgtgtttcctctcgccccctcctccaaaagcaccagcggaggaaccgctgctctcggatgtctggtgaaggactacttccctgaacccgtcaccgtgagctggaatagcggcgctctgacaagcggagtccatacattccctgctgtgctgcaaagcagcggactctattccctgtccagcgtcgtcacagtgcccagcagcagcctgggcacccagacctacatctgtaacgtcaaccacaagccctccaacaccaaggtggacaagaaagtggagcccaaatcctgcgacaagacacacacctgtcccccctgtcctgctcccgaagctgctggaggccctagcgtcttcctctttcctcccaaacccaaggacaccctcatgatcagcagaacccctgaagtcacctgtgtcgtcgtggatgtcagccatgaggaccccgaggtgaaattcaactggtatgtcgatggcgtcgaggtgcacaacgccaaaaccaagcccagggaggaacagtacaactccacctacagggtggtgtccgtgctgacagtcctccaccaggactggctgaacggcaaggagtacaagtgcaaggtgtccaacaaggctctccctgcccccattgagaagaccatcagcaaggccaaaggccaacccagggagccccaggtctatacactgcctccctccagggacgaactcaccaagaaccaggtgtccctgacctgcctggtcaagggcttttatcccagcgacatcgccgtcgagtgggagtccaacggacagcccgagaataactacaagaccacccctcctgtcctcgactccgacggctccttcttcctgtacagcaaactgaccgtcgataaatctaggtggcagcagggcaacgtgttctcttgttccgtgatgcatgaagcactgcacaaccattatacccagaagtctctgagcctgtcccccggcaagggcggcggcggctctggaggaggaggcagcggcggaggaggctccggaggcggcggctctgaggtgcagctggtggagtctggaggaggactggtgcagcctggaggctccctgaggctgtcttgcgcagcaagcggattcgcctttagctcctacgacatgagctgggtgcggcaggcacctggcaagggtctggattgggtggcaaccatcagcggaggcggcagatacacatactatcccgactccgtgaagggcaggttcaccatctcccgcgataactctaagaacaatctgtatctgcagatgaacagcctgagggccgaggacacagccctgtactattgcgccaaccgctacggcgaggcctggtttgcctattggggccagggcaccctggtgacagtgtctagcggcggcggcggcagcggcggcggcggctccggaggaggcggctctggcggcggcggcagcgatatccagatgacccagtccccctcctctatgtctgccagcgtgggcgaccgggtgaccttcacatgtagagcctcccaggatatcaacacctacctgtcttggtttcagcagaagcccggcaagagccctaagacactgatctatcgggccaatagactggtgagcggagtgccttcccggttctccggctctggcagcggacaggactataccctgacaatcagctccctgcagccagaggatatggccacatactattgcctgcagtatgacgagttccccctgaccttcggggctggcactaagctggagctgaaaaga

SEQ ID NO: 143 - protein, 214 aa, Artificial Sequence
  Synthetic artificial sequence-Amino acid sequence of VP101(hG1DM) light  chain
DIQMTQSPSSLSASVGDRVTITCSASQDISNYLNWYQQKPGKAPKVLIYFTSSLHSGVPSRFSGSGSGTDFTLTISSLQPEDFATYYCQQYSTVPWTFGQGTKVEIKRTVAAPSVFIFPPSDEQLKSGTASVVCLLNNFYPREAKVQWKVDNALQSGNSQESVTEQDSKDSTYSLSSTLTLSKADYEKHKVYACEVTHQGLSSPVTKSFNRGEC

SEQ ID NO: 144 - DNA, 642 bp, Artificial Sequence
  Synthetic artificial sequence-Nucleotide sequence of the light chain of VP101(hG1DM)
gatattcagatgactcagagcccctcctccctgtccgcctctgtgggcgacagggtcaccatcacatgcagtgcttcacaggatatttccaactacctgaattggtatcagcagaagccaggaaaagcacccaaggtgctgatctacttcactagctccctgcactcaggagtgccaagccggttcagcggatccggatctggaaccgactttactctgaccatttctagtctgcagcctgaggatttcgctacatactattgccagcagtattctaccgtgccatggacatttggccaggggactaaagtcgagatcaagcggaccgtggccgctcccagtgtcttcatttttccccctagcgacgaacagctgaaatccgggacagcctctgtggtctgtctgctgaacaacttctaccctagagaggcaaaagtgcagtggaaggtcgataacgccctgcagagtggcaattcacaggagagcgtgacagaacaggactccaaagattctacttatagtctgtcaagcacactgactctgagcaaggctgactacgaaaagcataaagtgtatgcatgtgaggtcacccaccaggggctgagcagtccagtcaccaagtcattcaacagaggcgagtgc

SEQ ID NO: 145 - DNA, 369 bp, Artificial Sequence
  Synthetic artificial sequence-Nucleotide sequence of the heavy chain variable region of Bevacizumab
gaggtgcagctggtcgagtccgggggggggctggtgcagccaggcgggtctctgaggctgagttgcgccgcttcagggtacaccttcacaaactatggaatgaattgggtgcgccaggcaccaggaaagggactggagtgggtcggctggatcaacacttacaccggggaacctacctatgcagccgactttaagcggcggttcaccttcagcctggatacaagcaaatccactgcctacctgcagatgaacagcctgcgagctgaggacaccgcagtctactattgtgctaaatatccccactactatgggagcagccattggtattttgacgtgtgggggcaggggactctggtgacagtgagcagc

SEQ ID NO: 146 - DNA, 321 bp, Artificial Sequence
  Synthetic artificial sequence-Nucleotide sequence of the variable region of the light chain of Bevacizumab
gatattcagatgactcagagcccctcctccctgtccgcctctgtgggcgacagggtcaccatcacatgcagtgcttcacaggatatttccaactacctgaattggtatcagcagaagccaggaaaagcacccaaggtgctgatctacttcactagctccctgcactcaggagtgccaagccggttcagcggatccggatctggaaccgactttactctgaccatttctagtctgcagcctgaggatttcgctacatactattgccagcagtattctaccgtgccatggacatttggccaggggactaaagtcgagatcaag